European Patent Application EP 4 124 347 A1, published February 1, 2023. Title: CIRCULAR RNA MOLECULE AND USE THEREOF IN TARGETED DEGRADATION OF PROTEIN OF INTEREST. Applicant: Suzhou Curemed Biomedical Technology Co. Ltd. The sequence listing filed with the application follows.

SEQUENCE LISTING (57 sequences)

SEQ ID NO: 1 - RNA, 2035 nt, synthetic construct
  misc_feature 1..2035: note = circular RNA molecule sequence
  source 1..2035: mol_type = other RNA
aaaatccgttgaccttaaacggtcgtgtgggttcaagtccctccacccccacgccggaaacgcaatagccgaaaaaacaaaaacaaaaaaaacaaaaaaacaaaaaaaaaaccaaaacacattaaaacagcctgtgggttgatcccacccacagggcccactgggcgctagcactctggtatcacggtacctttgtgcgcctgttttatacttcctcccccaactgcaacttagaagtaacacaaaccgatcaacagtcagcgtggcacaccagccacgttttgatcaaacacttctgttaccccggactgagtatcaatagactgctcacgcggttgaaggagaaaacgttcgttatccggccaactacttcgagaaacctagtaacgccatggaagttgtggagtgtttcgctcagcactaccccagtgtagatcaggttgatgagtcaccgcattccccacgggtgaccgtggcggtggctgcgttggcggcctgcccatggggaaacccatgggacgctcttatacagacatggtgcgaagagtctattgagctagttggtagtcctccggcccctgaatgcggctaatcccaactgcggagcatacactctcaagccagagggtagtgtgtcgtaatgggcaactctgcagcggaaccgactactttgggtgtccgtgtttcattttattcctatactggctgcttatggtgacaattgagagattgttaccatatagctattggattggccatccggtgactaacagagctattatatatctttttgttgggtttataccacttagcttgaaagaggttaaaactctacattacattttaatactgaacaccgcaaaatgcccgagcccgccaagagcgcccccgctcccaagaagggcagcaagaaggccgtgaccaaggcccagaagaagggcggcaagaaaaggaagaggagcaggaaggagagctacagcatctacgtgtacaaggtgctgaagcaggtgcaccccgacaccggcatcagcagcaaggccatgggcatcatgaacagcttcgtgaacgacatcttcgagaggatcgccggcgaggccagcagactggcccactacaacaagaggagcaccatcaccagcagagagatccagaccgccgtgagactgctgctgcccggcgagctggccaagcacgccgtgagcgagggcaccaaggccatcaccaagtacaccagcgccaaggaccctcccgtggccaccatggtgagcaagggcgaggagctgttcaccggcgtggtgcccatcctggtggagctggacggcgacgtgaacggccacaagttcagcgtgagcggcgagggagagggcgacgccacctacggcaagctgaccctgaagttcatctgcaccaccggcaagctgcccgtgccctggcccaccctggtgaccaccctgacctacggcgtgcagtgcttcagcaggtaccccgaccacatgaagcagcacgacttcttcaagagcgccatgcccgagggctacgtgcaggagaggaccatcttcttcaaggacgacggcaactacaagaccagggccgaggtgaagttcgagggcgacaccctggtgaacaggatcgagctgaagggcatcgacttcaaggaggacggcaacatcctgggccacaagctggagtacaactacaatagccacaacgtgtacatcatggccgacaagcagaagaacggcatcaaggtgaacttcaagatcaggcacaacatcgaggacggcagcgtgcagctggccgaccactaccagcagaacacccccatcggcgacggccccgtgctgctgcccgacaaccactacctgagcacccagagcgccctgagcaaggaccccaacgagaagagggaccacatggtgctgctggagttcgtgaccgccgccggcatcaccctgggcatggacgagctgtacaagtgaaaaaaacaaaaaacaaaacggctattatgcgttaccggcgagacgctacggactta

SEQ ID NO: 2 - RNA, 2089 nt, synthetic construct
  misc_feature 1..2089: note = circular RNA molecule sequence
  source 1..2089: mol_type = other RNA
aaaatccgttgaccttaaacggtcgtgtgggttcaagtccctccacccccacgccggaaacgcaatagccgaaaaaacaaaaacaaaaaaaacaaaaaaacaaaaaaaaaaccaaaacacattaaaacagcctgtgggttgatcccacccacagggcccactgggcgctagcactctggtatcacggtacctttgtgcgcctgttttatacttcctcccccaactgcaacttagaagtaacacaaaccgatcaacagtcagcgtggcacaccagccacgttttgatcaaacacttctgttaccccggactgagtatcaatagactgctcacgcggttgaaggagaaaacgttcgttatccggccaactacttcgagaaacctagtaacgccatggaagttgtggagtgtttcgctcagcactaccccagtgtagatcaggttgatgagtcaccgcattccccacgggtgaccgtggcggtggctgcgttggcggcctgcccatggggaaacccatgggacgctcttatacagacatggtgcgaagagtctattgagctagttggtagtcctccggcccctgaatgcggctaatcccaactgcggagcatacactctcaagccagagggtagtgtgtcgtaatgggcaactctgcagcggaaccgactactttgggtgtccgtgtttcattttattcctatactggctgcttatggtgacaattgagagattgttaccatatagctattggattggccatccggtgactaacagagctattatatatctttttgttgggtttataccacttagcttgaaagaggttaaaactctacattacattttaatactgaacaccgcaaaatgggcggcctggactacaaggacgacgacgataaggccagcagcgacctgggcaagaagctgctggaggccgccagggccggccaggacgacgaggtgaggatcctgatggccaacggcgccgacgtgaacgccctggacaggttcggcctgacccccttgcacctggccgcccagaggggccacctggagatcgtggaggtgctgctgaagtgcggcgccgacgtgaacgccgccgacctgtggggccagacccccttgcacctggctgccaccgccggccacctggagatcgtcgaggtgctgctgaagtacggcgccgacgtgaacgctctggacctgatcggcaagacccccttgcacctgaccgccatcgacggccacctggaaatcgtggaggtgctcctgaagcacggcgccgacgtgaacgcacaggacaagttcggcaagaccgcttttgatattagcatcgacaacggcaatgaggatcttgctgaaatcttgcagaagctgaacggctctggatctggcagcggaagcgtgaacatcagcggccagaacaccatgaacatggtgaaggtgcccgagtgcagactggccgacgagctgggcggcctgtgggagaacagcaggttcaccgactgctgcctgtgcgtggccggccaggagttccaggcccacaaggccatcctggccgccaggagccccgtgttcagcgccatgttcgagcacgagatggaggagagcaagaagaacagagtggagatcaacgacgtggagcccgaggtgttcaaggagatgatgtgcttcatctacaccggcaaggcccccaacctggacaagatggccgacgacctgctggccgccgccgacaagtacgccctggagagactgaaggtgatgtgcgaggacgccctgtgcagcaacctgagcgtggagaacgccgccgagatcctcatcctggccgacctgcacagcgccgaccagctgaagacccaggccgtggacttcatcaactaccacgccagcgacgtgctggagaccagcggctggaagagcatggtggtgagccacccccacctggtggccgaggcctacaggagcctggccagcgcccagtgccccttcctgggccctcccaggaagagactgaagcagagcggcagctgaaaaaaacaaaaaacaaaacggctattatgcgttaccggcgagacgctacggactta

SEQ ID NO: 3 - RNA, 1630 nt, synthetic construct
  misc_feature 1..1630: note = linear RNA molecule sequence
  source 1..1630: mol_type = other RNA
gactcactatttgttttcgcgcccagttgcaaaaagtgtcgcctagggttggccaatctactcccaggagcagggagggcaggagccagggctgggcataaaagtcagggcagagccatctattgcttacatttgcttctgacacaactgtgttcactagcaacctcaaacagacaccgccaccatgggcggcctggactacaaggacgacgacgataaggccagcagcgacctgggcaagaagctgctggaggccgccagggccggccaggacgacgaggtgaggatcctgatggccaacggcgccgacgtgaacgccctggacaggttcggcctgacccccttgcacctggccgcccagaggggccacctggagatcgtggaggtgctgctgaagtgcggcgccgacgtgaacgccgccgacctgtggggccagacccccttgcacctggctgccaccgccggccacctggagatcgtcgaggtgctgctgaagtacggcgccgacgtgaacgctctggacctgatcggcaagacccccttgcacctgaccgccatcgacggccacctggaaatcgtggaggtgctcctgaagcacggcgccgacgtgaacgcacaggacaagttcggcaagaccgcttttgatattagcatcgacaacggcaatgaggatcttgctgaaatcttgcagaagctgaacggctctggatctggcagcggaagcgtgaacatcagcggccagaacaccatgaacatggtgaaggtgcccgagtgcagactggccgacgagctgggcggcctgtgggagaacagcaggttcaccgactgctgcctgtgcgtggccggccaggagttccaggcccacaaggccatcctggccgccaggagccccgtgttcagcgccatgttcgagcacgagatggaggagagcaagaagaacagagtggagatcaacgacgtggagcccgaggtgttcaaggagatgatgtgcttcatctacaccggcaaggcccccaacctggacaagatggccgacgacctgctggccgccgccgacaagtacgccctggagagactgaaggtgatgtgcgaggacgccctgtgcagcaacctgagcgtggagaacgccgccgagatcctcatcctggccgacctgcacagcgccgaccagctgaagacccaggccgtggacttcatcaactaccacgccagcgacgtgctggagaccagcggctggaagagcatggtggtgagccacccccacctggtggccgaggcctacaggagcctggccagcgcccagtgccccttcctgggccctcccaggaagagactgaagcagagcggcagctgaagctcgctttcttgctgtccaatttctattaaaggttcctttgttccctaagtccaactactaaactgggggatattatgaagggccttgagcatctggattctgcctaataaaaaacatttattttcattgcgcatatgactagctcgctttcttgctgtccaatttctattaaaggttcctttgttccctaagtccaactactaaactgggggatattatgaagggccttgagcatctggattctgcctaataaaaaacatttattttcattgc

SEQ ID NO: 4 - RNA, 1648 nt, synthetic construct
  misc_feature 1..1648: note = circular RNA molecule sequence
  source 1..1648: mol_type = other RNA
aaaatccgttgaccttaaacggtcgtgtgggttcaagtccctccacccccacgccggaaacgcaatagccgaaaaaacaaaaacaaaaaaaacaaaaaaacaaaaaaaaaaccaaaacacattaaaacagcctgtgggttgatcccacccacagggcccactgggcgctagcactctggtatcacggtacctttgtgcgcctgttttatacttcctcccccaactgcaacttagaagtaacacaaaccgatcaacagtcagcgtggcacaccagccacgttttgatcaaacacttctgttaccccggactgagtatcaatagactgctcacgcggttgaaggagaaaacgttcgttatccggccaactacttcgagaaacctagtaacgccatggaagttgtggagtgtttcgctcagcactaccccagtgtagatcaggttgatgagtcaccgcattccccacgggtgaccgtggcggtggctgcgttggcggcctgcccatggggaaacccatgggacgctcttatacagacatggtgcgaagagtctattgagctagttggtagtcctccggcccctgaatgcggctaatcccaactgcggagcatacactctcaagccagagggtagtgtgtcgtaatgggcaactctgcagcggaaccgactactttgggtgtccgtgtttcattttattcctatactggctgcttatggtgacaattgagagattgttaccatatagctattggattggccatccggtgactaacagagctattatatatctttttgttgggtttataccacttagcttgaaagaggttaaaactctacattacattttaatactgaacaccgcaaaatggactacaaggacgacgacgataaggccagcagcgccgtgctgcagaagaagatcaccgactacttccaccccaagaagggcagcggctctggcagcggaagcgtgaacatcagcggccagaacaccatgaacatggtgaaggtgcccgagtgcagactggccgacgagctgggcggcctgtgggagaacagcaggttcaccgactgctgcctgtgcgtggccggccaggagttccaggcccacaaggccatcctggccgccaggagccccgtgttcagcgccatgttcgagcacgagatggaggagagcaagaagaacagagtggagatcaacgacgtggagcccgaggtgttcaaggagatgatgtgcttcatctacaccggcaaggcccccaacctggacaagatggccgacgacctgctggccgccgccgacaagtacgccctggagagactgaaggtgatgtgcgaggacgccctgtgcagcaacctgagcgtggagaacgccgccgagatcctcatcctggccgacctgcacagcgccgaccagctgaagacccaggccgtggacttcatcaactaccacgccagcgacgtgctggagaccagcggctggaagagcatggtggtgagccacccccacctggtggccgaggcctacaggagcctggccagcgcccagtgccccttcctgggccctcccaggaagagactgaagcagagctgaaaaaaacaaaaaacaaaacggctattatgcgttaccggcgagacgctacggactta

SEQ ID NO: 5 - RNA, 1648 nt, synthetic construct
  misc_feature 1..1648: note = circular RNA molecule sequence
  source 1..1648: mol_type = other RNA
aaaatccgttgaccttaaacggtcgtgtgggttcaagtccctccacccccacgccggaaacgcaatagccgaaaaaacaaaaacaaaaaaaacaaaaaaacaaaaaaaaaaccaaaacacattaaaacagcctgtgggttgatcccacccacagggcccactgggcgctagcactctggtatcacggtacctttgtgcgcctgttttatacttcctcccccaactgcaacttagaagtaacacaaaccgatcaacagtcagcgtggcacaccagccacgttttgatcaaacacttctgttaccccggactgagtatcaatagactgctcacgcggttgaaggagaaaacgttcgttatccggccaactacttcgagaaacctagtaacgccatggaagttgtggagtgtttcgctcagcactaccccagtgtagatcaggttgatgagtcaccgcattccccacgggtgaccgtggcggtggctgcgttggcggcctgcccatggggaaacccatgggacgctcttatacagacatggtgcgaagagtctattgagctagttggtagtcctccggcccctgaatgcggctaatcccaactgcggagcatacactctcaagccagagggtagtgtgtcgtaatgggcaactctgcagcggaaccgactactttgggtgtccgtgtttcattttattcctatactggctgcttatggtgacaattgagagattgttaccatatagctattggattggccatccggtgactaacagagctattatatatctttttgttgggtttataccacttagcttgaaagaggttaaaactctacattacattttaatactgaacaccgcaaaatggactacaaggacgacgacgataaggccagcagcgccgtgctgcagaagaaggccaccgacgccgcccaccccaagaagggcagcggctctggcagcggaagcgtgaacatcagcggccagaacaccatgaacatggtgaaggtgcccgagtgcagactggccgacgagctgggcggcctgtgggagaacagcaggttcaccgactgctgcctgtgcgtggccggccaggagttccaggcccacaaggccatcctggccgccaggagccccgtgttcagcgccatgttcgagcacgagatggaggagagcaagaagaacagagtggagatcaacgacgtggagcccgaggtgttcaaggagatgatgtgcttcatctacaccggcaaggcccccaacctggacaagatggccgacgacctgctggccgccgccgacaagtacgccctggagagactgaaggtgatgtgcgaggacgccctgtgcagcaacctgagcgtggagaacgccgccgagatcctcatcctggccgacctgcacagcgccgaccagctgaagacccaggccgtggacttcatcaactaccacgccagcgacgtgctggagaccagcggctggaagagcatggtggtgagccacccccacctggtggccgaggcctacaggagcctggccagcgcccagtgccccttcctgggccctcccaggaagagactgaagcagagctgaaaaaaacaaaaaacaaaacggctattatgcgttaccggcgagacgctacggactta

SEQ ID NO: 6 - RNA, 1573 nt, synthetic construct
  misc_feature 1..1573: note = circular RNA molecule sequence
  source 1..1573: mol_type = other RNA
aaaatccgttgaccttaaacggtcgtgtgggttcaagtccctccacccccacgccggaaacgcaatagccgaaaaaacaaaaacaaaaaaaacaaaaaaacaaaaaaaaaaccaaaacacattaaaacagcctgtgggttgatcccacccacagggcccactgggcgctagcactctggtatcacggtacctttgtgcgcctgttttatacttcctcccccaactgcaacttagaagtaacacaaaccgatcaacagtcagcgtggcacaccagccacgttttgatcaaacacttctgttaccccggactgagtatcaatagactgctcacgcggttgaaggagaaaacgttcgttatccggccaactacttcgagaaacctagtaacgccatggaagttgtggagtgtttcgctcagcactaccccagtgtagatcaggttgatgagtcaccgcattccccacgggtgaccgtggcggtggctgcgttggcggcctgcccatggggaaacccatgggacgctcttatacagacatggtgcgaagagtctattgagctagttggtagtcctccggcccctgaatgcggctaatcccaactgcggagcatacactctcaagccagagggtagtgtgtcgtaatgggcaactctgcagcggaaccgactactttgggtgtccgtgtttcattttattcctatactggctgcttatggtgacaattgagagattgttaccatatagctattggattggccatccggtgactaacagagctattatatatctttttgttgggtttataccacttagcttgaaagaggttaaaactctacattacattttaatactgaacaccgcaaaatggactacaaggacgacgacgataaggccagcagcgccgtgctgcagaagaagatcaccgactacttccaccccaagaagggcagcggctctggcagcggaagcgtgaacatcagcggccagaacaccatgaacatggtgaaggtgcccgagtgcagactggccgacgagctgggcggcctgtgggagaacagcaggttcaccgactgctgcctgtgcgtggccggccaggagttccaggcccacaaggccatcctggccgccaggagccccgtgttcagcgccatgttcgagcacgagatggaggagagcaagaagaacagagtggagatcaacgacgtggagcccgaggtgttcaaggagatgatgtgcttcatctacaccggcaaggcccccaacctggacaagatggccgacgacctgctggccgccgccgacaagtacgccctggagagactgaaggtgatgtgcgaggacgccctgtgcagcaacctgagcgtggagaactaccacgccagcgacgtgctggagaccagcggctggaagagcatggtggtgagccacccccacctggtggccgaggcctacaggagcctggccagcgcccagtgccccttcctgggccctcccaggaagagactgaagcagagctgaaaaaaacaaaaaacaaaacggctattatgcgttaccggcgagacgctacggactta

SEQ ID NO: 7 - protein, 261 aa, Homo sapiens
MFEARLVQGSILKKVLEALKDLINEACWDISSSGVNLQSMDSSHVSLVQLTLRSEGFDTYRCDRNLAMGVNLTSMSKILKCAGNEDIITLRAEDNADTLALVFEAPNQEKVSDYEMKLMDLDVEQLGIPEQEYSCVVKMPSGEFARICRDLSHIGDAVVISCAKDGVKFSASGELGNGNIKLSQTSNVDKEEEAVTIEMNEPVQLTFALRYLNFFTKATPLSSTVTLSMSADVPLVVEYKIADMGHLKYYLAPKIEDEEGS

SEQ ID NO: 8 - protein, 16 aa, synthetic construct
  REGION 1..16: note = first polypeptide sequence
SAVLQKKITDYFHPKK

SEQ ID NO: 9 - DNA, 48 bp, synthetic construct
  misc_feature 1..48: note = first polypeptide sequence
  source 1..48: mol_type = other DNA
agcgccgtgctgcagaagaagatcaccgactacttccaccccaagaag

SEQ ID NO: 10 - protein, 7 aa, synthetic construct
  REGION 1..7: note = linker peptide sequence
GSGSGSG

SEQ ID NO: 11 - DNA, 21 bp, synthetic construct
  misc_feature 1..21: note = linker peptide sequence
  source 1..21: mol_type = other DNA
ggcagcggctctggcagcgga

SEQ ID NO: 12 - protein, 208 aa, synthetic construct
  REGION 1..208: note = second polypeptide sequence
SVNISGQNTMNMVKVPECRLADELGGLWENSRFTDCCLCVAGQEFQAHKAILAARSPVFSAMFEHEMEESKKNRVEINDVEPEVFKEMMCFIYTGKAPNLDKMADDLLAAADKYALERLKVMCEDALCSNLSVENAAEILILADLHSADQLKTQAVDFINYHASDVLETSGWKSMVVSHPHLVAEAYRSLASAQCPFLGPPRKRLKQS

SEQ ID NO: 13 - DNA, 627 bp, synthetic construct
  misc_feature 1..627: note = second polypeptide sequence
  source 1..627: mol_type = other DNA
agcgtgaacatcagcggccagaacaccatgaacatggtgaaggtgcccgagtgcagactggccgacgagctgggcggcctgtgggagaacagcaggttcaccgactgctgcctgtgcgtggccggccaggagttccaggcccacaaggccatcctggccgccaggagccccgtgttcagcgccatgttcgagcacgagatggaggagagcaagaagaacagagtggagatcaacgacgtggagcccgaggtgttcaaggagatgatgtgcttcatctacaccggcaaggcccccaacctggacaagatggccgacgacctgctggccgccgccgacaagtacgccctggagagactgaaggtgatgtgcgaggacgccctgtgcagcaacctgagcgtggagaacgccgccgagatcctcatcctggccgacctgcacagcgccgaccagctgaagacccaggccgtggacttcatcaactaccacgccagcgacgtgctggagaccagcggctggaagagcatggtggtgagccacccccacctggtggccgaggcctacaggagcctggccagcgcccagtgccccttcctgggccctcccaggaagagactgaagcagagctga

SEQ ID NO: 14 - RNA, 741 nt, synthetic construct
  misc_feature 1..741: note = IRES sequence
  source 1..741: mol_type = other RNA
ttaaaacagcctgtgggttgatcccacccacaggcccattgggcgctagcactctggtatcacggtacctttgtgcgcctgttttataccccctcccccaactgtaacttagaagtaacacacaccgatcaacagtcagcgtggcacaccagccacgttttgatcaagcacttctgttaccccggactgagtatcaatagactgctcacgcggttgaaggagaaagcgttcgttatccggccaactacttcgaaaaacctagtaacaccgtggaagttgcagagtgtttcgctcagcactaccccagtgtagatcaggtcgatgagtcaccgcattccccacgggcgaccgtggcggtggctgcgttggcggcctgcccatggggaaacccatgggacgctctaatacagacatggtgcgaagagtctattgagctagttggtagtcctccggcccctgaatgcggctaatcctaactgcggagcacacaccctcaagccagagggcagtgtgtcgtaacgggcaactctgcagcggaaccgactactttgggtgtccgtgtttcattttattcctatactggctgcttatggtgacaattgagagatcgttaccatatagctattggattggccatccggtgactaatagagctattatatatccctttgttgggtttataccacttagcttgaaagaggttaaaacattacaattcattgttaagttgaatacagcaaa

SEQ ID NO: 15 - RNA, 682 nt, synthetic construct
  misc_feature 1..682: note = IRES sequence
  source 1..682: mol_type = other RNA
ttaaaacagcctgtgggttgcacccacccacagggcccacagggcgctagcactctggtatcacggtacctttgtgcgcctgttttattaccccttccccaattgaaaattagaagcaatgcacaccgatcaacagcaggcgtggcgcaccagtcacgtctcgatcaagcacttctgtttccccggaccgagtatcaatagactgctcacgcggttgaaggagaaagtgttcgttatccggctaaccacttcgagaaacccagtaacaccatgaaagttgcagggtgtttcgctcagcacttccccagtgtagatcaggtcgatgagtcaccgcgttccccacgggcgaccgtggcggtggctgcgttggcggcctgcctatgggttaacccataggacgctctaatacagacatggtgcgaagagtttattgagctggttagtatccctccggcccctgaatgcggctaatcctaactgcggagcacgtgcctccaatccagggggttgcatgtcgtaacgggtaactctgcagcggaaccgactactttgggtgtccgtgtttccttttattcttatactggctgcttatggtgacaatcgaggaattgttaccatatagctattggattggccatccggtgtctaacagagcgattatatacctctttgttggatttat

SEQ ID NO: 16 - RNA, 742 nt, synthetic construct
  misc_feature 1..742: note = IRES sequence
  source 1..742: mol_type = other RNA
ttaaaacagcctgtgggttgatcccacccacagggcccactgggcgctagcactctggtatcacggtacctttgtgcgcctgttttatacttcctcccccaactgcaacttagaagtaacacaaaccgatcaacagtcagcgtggcacaccagccacgttttgatcaaacacttctgttaccccggactgagtatcaatagactgctcacgcggttgaaggagaaaacgttcgttatccggccaactacttcgagaaacctagtaacgccatggaagttgtggagtgtttcgctcagcactaccccagtgtagatcaggttgatgagtcaccgcattccccacgggtgaccgtggcggtggctgcgttggcggcctgcccatggggaaacccatgggacgctcttatacagacatggtgcgaagagtctattgagctagttggtagtcctccggcccctgaatgcggctaatcccaactgcggagcatacactctcaagccagagggtagtgtgtcgtaatgggcaactctgcagcggaaccgactactttgggtgtccgtgtttcattttattcctatactggctgcttatggtgacaattgagagattgttaccatatagctattggattggccatccggtgactaacagagctattatatatctttttgttgggtttataccacttagcttgaaagaggttaaaactctacattacattttaatactgaacaccgcaaa

SEQ ID NO: 17 - RNA, 737 nt, synthetic construct
  misc_feature 1..737: note = IRES sequence
  source 1..737: mol_type = other RNA
ttaaaacagcctgtgggttgatcccacccacagggcccattgggcgctagcactctggtatcacggtacccttgtgcgcctgttttatgtcccttccctcaactgtaacttagaagtaacgcacaccgatcaacagtcagcgtggcacaccagccatgttttgatcaagcacttctgttaccccggaccgagtatcaacagactgctcacgcggttgaaggagaaagtgttcgttatccggccaactacttcgaaaaacctagtaacaccatggaagttgcagagtgtttcgctcagcactaccccagtgtagatcaggtcgatgagtcaccgcatcccccacgggcgaccgtggcggtggctgcgttggcggcctgcctatgggggaacccataggacgctctaatacagacatggtgcgaagagtccattgagctagttggtagtcctccggcccctgaatgcggctaatcctaactgcggagcacacaccttcaagccagagggcagtgtgtcgtaacgggcaactctgcagcggaaccgactactttgggtgtccgtgtttcattttattcttatactggctgcttatggtgacaattgagagattgttaccatatagctattggattggccatccagtgactagcagagctattatatacctctttgttgggtttataccacctaatttgaaagaagttaaaacattagaattcattattaaattgaataca

SEQ ID NO: 18 - RNA, 683 nt, synthetic construct
  misc_feature 1..683: note = IRES sequence
  source 1..683: mol_type = other RNA
ttaaaacagcctgtgggttgcacccacccacagggcccacagggcgctagcactctggtatcacggtacctttgtgcgcctgttttattaccccttccccaattgaaaattagaagcaatgcacaccgatcaacagcaggcgtggcgcaccagtcacgtctcgatcaagcacttctgtttccccggaccgagtatcaatagactgctcacgcggttgaaggagaaagtgttcgttatccggctaaccacttcgagaaacccagtaacaccatgaaagttgcagggtgtttcgctcagcacttccccagtgtagatcaggtcgatgagtcaccgcgttccccacgggcgaccgtggcggtggctgcgttggcggcctgcctatgggttaacccataggacgctctaatacagacatggtgcgaagagtttattgagctggttagtatctcctccggcccctgaatgcggctaatcctaactgcggagcacacaccctcaagccagagggcagtgtgtcgtaacgggcaactctgcagcggaaccgactactttgggtgtccgtgtttccttttattcttatactggctgcttatggtgacaatcgaggaattgttaccatatagctattggattggccatccggtgtctaacagagcgattatatacctctttgttggatttat

SEQ ID NO: 19 - RNA, 742 nt, synthetic construct
  misc_feature 1..742: note = IRES sequence
  source 1..742: mol_type = other RNA
ttaaaacagcctgtgggttgatcccacccacagggcccactgggcgctagcactctggtatcacggtacctttgtgcgcctgttttatacttcctcccccaactgcaacttagaagtaacacaaaccgatcaacagtcagcgtggcacaccagccacgttttgatcaaacacttctgttaccccggactgagtatcaatagactgctcacgcggttgaaggagaaaacgttcgttatccggccaactacttcgagaaacctagtaacgccatggaagttgtggagtgtttcgctcagcactaccccagtgtagatcaggttgatgagtcaccgcattccccacgggtgaccgtggcggtggctgcgttggcggcctgcccatggggaaacccatgggacgctcttatacagacatggtgcgaagagtctattgagctagttggtagtcctccggcccctgaatgcggctaatcctaactgcggagcacacaccctcaagccagagggcagtgtgtcgtaacgggcaactctgcagcggaaccgactactttgggtgtccgtgtttcattttattcctatactggctgcttatggtgacaattgagagattgttaccatatagctattggattggccatccggtgactaacagagctattatatatctttttgttgggtttataccacttagcttgaaagaggttaaaactctacattacattttaatactgaacaccgcaaa

SEQ ID NO: 20 - RNA, 737 nt, synthetic construct
  misc_feature 1..737: note = IRES sequence
  source 1..737: mol_type = other RNA
ttaaaacagcctgtgggttgatcccacccacagggcccattgggcgctagcactctggtatcacggtacccttgtgcgcctgttttatgtcccttccctcaactgtaacttagaagtaacgcacaccgatcaacagtcagcgtggcacaccagccatgttttgatcaagcacttctgttaccccggaccgagtatcaacagactgctcacgcggttgaaggagaaagtgttcgttatccggccaactacttcgaaaaacctagtaacaccatggaagttgcagagtgtttcgctcagcactaccccagtgtagatcaggtcgatgagtcaccgcatcccccacgggcgaccgtggcggtggctgcgttggcggcctgcctatgggggaacccataggacgctctaatacagacatggtgcgaagagtccattgagctagttggtagtcctccggcccctgaatgcggctaatcctaactgcggagcacacaccctcaagccagagggcagtgtgtcgtaacgggcaactctgcagcggaaccgactactttgggtgtccgtgtttcattttattcttatactggctgcttatggtgacaattgagagattgttaccatatagctattggattggccatccagtgactagcagagctattatatacctctttgttgggtttataccacctaatttgaaagaagttaaaacattagaattcattattaaattgaataca

SEQ ID NO: 21 - RNA, 16 nt, synthetic construct
  misc_feature 1..16: note = first exon sequence
  source 1..16: mol_type = other RNA
agacgctacggactta

SEQ ID NO: 22 - RNA, 51 nt, synthetic construct
  misc_feature 1..51: note = second exon sequence
  source 1..51: mol_type = other RNA
aaaatccgttgaccttaaacggtcgtgtgggttcaagtccctccaccccca

SEQ ID NO: 23 - RNA, 50 nt, synthetic construct
  misc_feature 1..50: note = 5' spacer sequence
  source 1..50: mol_type = other RNA
aaaaaacaaaaacaaaaaaaacaaaaaaacaaaaaaaaaaccaaaacaca

SEQ ID NO: 24 - RNA, 50 nt, synthetic construct
  misc_feature 1..50: note = 5' spacer sequence
  source 1..50: mol_type = other RNA
aaaaacaaaaaacaaaaaaaaaaccaaaaaaacaaaaaaaacaaaacaca

SEQ ID NO: 25 - RNA, 25 nt, synthetic construct
  misc_feature 1..25: note = 3' spacer sequence
  source 1..25: mol_type = other RNA
aaaaaaacaaaaaaacaaaacaaac

SEQ ID NO: 26 - RNA, 22 nt, synthetic construct
  misc_feature 1..22: note = 3' spacer sequence
  source 1..22: mol_type = other RNA
aaaaacaaaaaacaaaacaaac

SEQ ID NO: 27 - DNA, 114 bp, synthetic construct
  misc_feature 1..114: note = 5' intron sequence
  source 1..114: mol_type = other DNA
aataattgagccttaaagaagaaattctttaagtggatgctctcaaactcagggaaacctaaatctagttatagacaaggcaatcctgagccaagccgaagtagtaattagtaa

SEQ ID NO: 28 - DNA, 131 bp, synthetic construct
  misc_feature 1..131: note = 3' intron sequence
  source 1..131: mol_type = other DNA
aacaatagatgacttacaactaatcggaaggtgcagagactcgacgggagctaccctaacgtcaagacgagggtaaagagagagtccaattctcaaagccaataggcagtagcgaaagctgcaagagaatg

SEQ ID NO: 29 - DNA, 21 bp, synthetic construct
  misc_feature 1..21: note = 5' homologous arm sequence
  source 1..21: mol_type = other DNA
accgtcagttgctcactgtgc

SEQ ID NO: 30 - DNA, 21 bp, synthetic construct
  misc_feature 1..21: note = 5' homologous arm sequence
  source 1..21: mol_type = other DNA
accgtgctatgtccacgtgtc

SEQ ID NO: 31 - DNA, 21 bp, synthetic construct
  misc_feature 1..21: note = 3' homologous arm sequence
  source 1..21: mol_type = other DNA
gcacagtgagcaactgacgga

SEQ ID NO: 32 - DNA, 21 bp, synthetic construct
  misc_feature 1..21: note = 3' homologous arm sequence
  source 1..21: mol_type = other DNA
gacacgtggacatagcacgga

SEQ ID NO: 33 - protein, 170 aa, synthetic construct
  REGION 1..170: note = first peptide sequence
MDLGKKLLEAARAGQDDEVRILMANGADVNASDRGGGTPLHLAAAGGHLEIVEVLLKRGADVSAADLHGQSPLHLAAMVGHLEIVEVLLKYGADVNAKDTMGATPLHLAARSGHLEIVEELLKNGADMNAQDKFGKTTFDISTDNGNEDLAEILQKLVDGGSDYKDDDDK

SEQ ID NO: 34 - protein, 387 aa, synthetic construct
  REGION 1..387: note = recombinant peptide sequence
MGGLDYKDDDDKASSDLGKKLLEAARAGQDDEVRILMANGADVNALDRFGLTPLHLAAQRGHLEIVEVLLKCGADVNAADLWGQTPLHLAATAGHLEIVEVLLKYGADVNALDLIGKTPLHLTAIDGHLEIVEVLLKHGADVNAQDKFGKTAFDISIDNGNEDLAEILQKLNGSGSGSGSVNISGQNTMNMVKVPECRLADELGGLWENSRFTDCCLCVAGQEFQAHKAILAARSPVFSAMFEHEMEESKKNRVEINDVEPEVFKEMMCFIYTGKAPNLDKMADDLLAAADKYALERLKVMCEDALCSNLSVENAAEILILADLHSADQLKTQAVDFINYHASDVLETSGWKSMVVSHPHLVAEAYRSLASAQCPFLGPPRKRLKQS

SEQ ID NO: 35 - protein, 242 aa, synthetic construct
  REGION 1..242: note = recombinant peptide sequence
MDYKDDDDKASSAVLQKKITDYFHPKKGSGSGSGSVNISGQNTMNMVKVPECRLADELGGLWENSRFTDCCLCVAGQEFQAHKAILAARSPVFSAMFEHEMEESKKNRVEINDVEPEVFKEMMCFIYTGKAPNLDKMADDLLAAADKYALERLKVMCEDALCSNLSVENAAEILILADLHSADQLKTQAVDFINYHASDVLETSGWKSMVVSHPHLVAEAYRSLASAQCPFLGPPRKRLKQS

SEQ ID NO: 36 - protein, 441 aa, synthetic construct
  REGION 1..441: note = recombinant peptide sequence
MGGLDYKDDDDKASDPAEAVLQEKALKFMNSSEREDCNNGEPPRKIIPEKNSLRQTYNSCARLCLNQETVCLASTAMKTENCVAKTKLANGTSSMIVPKQRKLSASYEKEKELCVKYFEQWSESDQVEFVEHLISQMCHYQHGHINSYLKPMLQRDFITALPARGLDHIAENILSYLDAKSLCAAELVCKEWYRVTSDGMLWKKLIERMVRTDSLWRGLAERRGWGQYLFKNKPPDGNAPPNSFYRALYPKIIQDIETIESNWRCGRHSLQRIHCRSGSGSGSGMDLGKKLLEAARAGQDDEVRILMANGADVNASDRGGGTPLHLAAAGGHLEIVEVLLKRGADVSAADLHGQSPLHLAAMVGHLEIVEVLLKYGADVNAKDTMGATPLHLAARSGHLEIVEELLKNGADMNAQDKFGKTTFDISTDNGNEDLAEILQKL

SEQ ID NO: 37 - protein, 471 aa, synthetic construct
  REGION 1..471: note = recombinant peptide sequence
MGGLDYKDDDDKASCVPRSGLILSCICLYCGVLLPVLLPNLPFLTCLSMSTLESVTYLPEKGLYCQRLPSSRTHGGTESLKGKNTENMGFYGTLKMIFYKMKRKLDHGSEVRSFSLGKKPCKVSEYTSTTGLVPCSATPTTFGDLRAANGQGQQRRRITSVQPPTGLQEWLKMFQSWSGPEKLLALDELIDSCEPTQVKHMMQVIEPQFQRDFISLLPKELALYVLSFLEPKDLLQAAQTCRYWRILAEDNLLWREKCKEEGIDEPLHIKRRKVIKPGFIHSPWKSAYIRQHRIDTNWRRGELKSPSGSGSGSGMDLGKKLLEAARAGQDDEVRILMANGADVNASDRGGGTPLHLAAAGGHLEIVEVLLKRGADVSAADLHGQSPLHLAAMVGHLEIVEVLLKYGADVNAKDTMGATPLHLAARSGHLEIVEELLKNGADMNAQDKFGKTTFDISTDNGNEDLAEILQKL

SEQ ID NO: 38 - protein, 325 aa, synthetic construct
  REGION 1..325: note = recombinant peptide sequence
MGGLDYKDDDDKASHRKHLQEIPDLSSNVATSFTWGWDSSKTSELLSGMGVSALEKEEPDSENIPQELLSNLGHPESPPRKRLKSKGSDKDFVIVRRPKLNRENFPGVSWDSLPDELLLGIFSCLCLPELLKVSGVCKRWYRLASDESLWQTLDLTGKNLSGSGSGSGMDLGKKLLEAARAGQDDEVRILMANGADVNASDRGGGTPLHLAAAGGHLEIVEVLLKRGADVSAADLHGQSPLHLAAMVGHLEIVEVLLKYGADVNAKDTMGATPLHLAARSGHLEIVEELLKNGADMNAQDKFGKTTFDISTDNGNEDLAEILQKL

SEQ ID NO: 39 - protein, 498 aa, synthetic construct
  REGION 1..498: note = recombinant peptide sequence
MGGLDYKDDDDKASAGEGDQQDAAHNMGNHLPLLPAESEEEDEMEVEDQDSKEAKKPNIINFDTSLPTSHTYLGADMEEFHGRTLHDDDSCQVIPVLPQVMMILIPGQTLPLQLFHPQEVSMVRNLIQKDRTFAVLAYSNVQEREAQFGTTAEIYAYREEQDFGIEIVKVKAIGRQRFKVLELRTQSDGIQQAKVQILPECVLPSTMSAVQLESLNKCQIFPSKPVSREDQCSYKWWQKYQKRKFHCANLTSWPRWLYSLYDAETLMDRIKKQLREWDENLKDDSLPSNPIDFSYRVAACLPIDDVLRIQLLKIGSAIQRLRCELDIMNKCTSSGSGSGSGMDLGKKLLEAARAGQDDEVRILMANGADVNASDRGGGTPLHLAAAGGHLEIVEVLLKRGADVSAADLHGQSPLHLAAMVGHLEIVEVLLKYGADVNAKDTMGATPLHLAARSGHLEIVEELLKNGADMNAQDKFGKTTFDISTDNGNEDLAEILQKL

SEQ ID NO: 40 - protein, 292 aa, synthetic construct
  REGION 1..292: note = recombinant peptide sequence
MGGLDYKDDDDKASAPKKRPETQKTSEIVLRPRNKRSRSPLELEPEAKKLCAKGSGPSRRCDSDCLWVGLAGPQILPPCRSIVRTLHQHKLGRASWPSVQQGLQQSFLHTLDSYRILQKAAPFDRRASGSGSGSGMDLGKKLLEAARAGQDDEVRILMANGADVNASDRGGGTPLHLAAAGGHLEIVEVLLKRGADVSAADLHGQSPLHLAAMVGHLEIVEVLLKYGADVNAKDTMGATPLHLAARSGHLEIVEELLKNGADMNAQDKFGKTTFDISTDNGNEDLAEILQKL

SEQ ID NO: 41 - protein, 223 aa, synthetic construct
  REGION 1..223: note = recombinant peptide sequence
MDLGKKLLEAARAGQDDEVRILMANGADVNASDRGGGTPLHLAAAGGHLEIVEVLLKRGADVSAADLHGQSPLHLAAMVGHLEIVEVLLKYGADVNAKDTMGATPLHLAARSGHLEIVEELLKNGADMNAQDKFGKTTFDISTDNGNEDLAEILQKLSGSGSGSGPRNGTVHLYLTKPLYTSAPSLQHLCRLTINKCTGAIWGLPLPTRLKDYLEEYKFQVGS

SEQ ID NO: 42 - protein, 237 aa, synthetic construct
  REGION 1..237: note = recombinant peptide sequence
MDLGKKLLEAARAGQDDEVRILMANGADVNASDRGGGTPLHLAAAGGHLEIVEVLLKRGADVSAADLHGQSPLHLAAMVGHLEIVEVLLKYGADVNAKDTMGATPLHLAARSGHLEIVEELLKNGADMNAQDKFGKTTFDISTDNGNEDLAEILQKLSGSGSGSGVKWESLGPESRGRRKVDPEALQVFKEARSVPRTLLCLCRVAVRRALGKHRLHLIPSLPLPDPIKKFLLHEGS

SEQ ID NO: 43 - protein, 343 aa, synthetic construct
  REGION 1..343: note = recombinant peptide sequence
MDLGKKLLEAARAGQDDEVRILMANGADVNASDRGGGTPLHLAAAGGHLEIVEVLLKRGADVSAADLHGQSPLHLAAMVGHLEIVEVLLKYGADVNAKDTMGATPLHLAARSGHLEIVEELLKNGADMNAQDKFGKTTFDISTDNGNEDLAEILQKLSGSGSGSGRLNFGDDIPSALRIAKKKRWNSIEERRIHQESELHSYLSRLIAAERERELEECQRNHEGDEDDSHVRAQQACIEAKHDKYMADMDELFSQVDEKRKKRDIPDYLCGKISFELMREPCITPSGITYDRKDIEEHLQRVGHFDPVTRSPLTQEQLIPNLAMKEVIDAFISENGWVEDYGS

SEQ ID NO: 44 - protein, 372 aa, synthetic construct
  REGION 1..372: note = recombinant peptide sequence
MDLGKKLLEAARAGQDDEVRILMANGADVNASDRGGGTPLHLAAAGGHLEIVEVLLKRGADVSAADLHGQSPLHLAAMVGHLEIVEVLLKYGADVNAKDTMGATPLHLAARSGHLEIVEELLKNGADMNAQDKFGKTTFDISTDNGNEDLAEILQKLGSGSGSGSVNISGQNTMNMVKVPECRLADELGGLWENSRFTDCCLCVAGQEFQAHKAILAARSPVFSAMFEHEMEESKKNRVEINDVEPEVFKEMMCFIYTGKAPNLDKMADDLLAAADKYALERLKVMCEDALCSNLSVENAAEILILADLHSADQLKTQAVDFINYHASDVLETSGWKSMVVSHPHLVAEAYRSLASAQCPFLGPPRKRLKQS

SEQ ID NO: 45 - protein, 393 aa, synthetic construct
  REGION 1..393: note = recombinant peptide sequence
MPRRAENWDEAEVGAEEAGVEEYGPEEDGGEESGAEESGPEESGPEELGAEEEMEAGRPRPVLRSVNSREPSQVIFCNRSPRVVLPVWLNFDGEPQPYPTLPPGTGRRIHSYRGHLWLFRDAGTHDGLLVNQTELFVPSLNVDGQPIFANITLPVYTLKERCLQVVRSLVKPENYRRLDIVRSLYEDLEDHPNVQKDLERLTQERIAHQRMGDLEGGGGSAAAMDLGKKLLEAARAGQDDEVRILMANGADVNASDRWGWTPLHLAAWWGHLEIVEVLLKRGADVSAADLHGQSPLHLAAMVGHLEIVEVLLKYGADVNAKDTMGATPLHLAARSGHLEIVEELLKNGADMNAQDKFGKTTFDISTDNGNEDLAEILQKLVDGGSDYKDDDDK

SEQ ID NO: 46 - RNA, 2245 nt, synthetic construct
  misc_feature 1..2245: note = circular RNA molecule sequence
  source 1..2245: mol_type = other RNA
aaaatccgttgaccttaaacggtcgtgtgggttcaagtccctccacccccacgccggaaacgcaatagccgaaaaaacaaaaacaaaaaaaacaaaaaaacaaaaaaaaaaccaaaacacattaaaacagcctgtgggttgatcccacccacagggcccactgggcgctagcactctggtatcacggtacctttgtgcgcctgttttatacttcctcccccaactgcaacttagaagtaacacaaaccgatcaacagtcagcgtggcacaccagccacgttttgatcaaacacttctgttaccccggactgagtatcaatagactgctcacgcggttgaaggagaaaacgttcgttatccggccaactacttcgagaaacctagtaacgccatggaagttgtggagtgtttcgctcagcactaccccagtgtagatcaggttgatgagtcaccgcattccccacgggtgaccgtggcggtggctgcgttggcggcctgcccatggggaaacccatgggacgctcttatacagacatggtgcgaagagtctattgagctagttggtagtcctccggcccctgaatgcggctaatcccaactgcggagcatacactctcaagccagagggtagtgtgtcgtaatgggcaactctgcagcggaaccgactactttgggtgtccgtgtttcattttattcctatactggctgcttatggtgacaattgagagattgttaccatatagctattggattggccatccggtgactaacagagctattatatatctttttgttgggtttataccacttagcttgaaagaggttaaaactctacattacattttaatactgaacaccgcaaaatgggcggcctggactacaaggatgacgacgacaaggccagcgaccccgccgaggccgtgctgcaggagaaggccctgaagttcatgaacagcagcgagagggaggactgcaacaacggcgagccccctaggaagatcatccccgagaagaacagcctgaggcagacctacaacagctgcgccaggctgtgcctgaaccaggagaccgtgtgcctggccagcaccgccatgaagaccgagaactgcgtggccaagaccaagctggccaacggcaccagcagcatgatcgtgcccaagcagaggaagctgagcgccagctacgagaaagagaaggagctgtgcgtgaagtacttcgagcagtggagcgagtccgaccaggtggagttcgtggagcacctgatcagccagatgtgccactaccagcacggccacatcaacagctacctgaagcccatgctgcagagggacttcatcaccgccctgcccgccaggggcctggaccacatcgccgagaacatcctgagctacctggacgccaagagcctgtgcgccgccgagctggtgtgcaaggagtggtacagggtgaccagcgacggcatgctgtggaagaagctgatcgagaggatggtgaggaccgacagcctgtggaggggcctggccgagaggaggggctggggccagtacctgttcaagaacaagccccctgacggcaacgcccctcccaacagcttctacagggccctgtaccccaagatcatccaggacatcgagaccatcgagtctaactggaggtgcggcaggcacagcctgcagaggatccactgcaggagcggcagcgggagcggcagcgggatggacctgggcaagaagctgctggaggccgccagggccggccaggacgacgaggtgaggatcctgatggccaacggcgccgatgtgaacgcttctgacaggggaggaggaacccctttacacctggccgccgccggaggccacctggagatcgtggaggtgctgttgaagaggggagctgacgtgagcgctgctgacctgcacggccagagccccttgcaccttgctgccatggtgggacacctggagatcgtggaagtgctgttgaagtacggcgctgacgtgaacgccaaggacaccatgggcgccacccccttgcacctggccgccaggtctggacacttagagatcgtggaggagctgctgaagaacggcgccgacatgaacgcccaggacaagttcggcaagaccaccttcgacatcagcaccgacaacggcaacgaggacctggccgagatcctgcagaagctgtgaaaaaaacaaaaaacaaaacggctattatgcgttaccggcgagacgctacggactta

SEQ ID NO: 47 - RNA, 2335 nt, synthetic construct
  misc_feature 1..2335: note = circular RNA molecule sequence
  source 1..2335: mol_type = other RNA
aaaatccgttgaccttaaacggtcgtgtgggttcaagtccctccacccccacgccggaaacgcaatagccgaaaaaacaaaaacaaaaaaaacaaaaaaacaaaaaaaaaaccaaaacacattaaaacagcctgtgggttgatcccacccacagggcccactgggcgctagcactctggtatcacggtacctttgtgcgcctgttttatacttcctcccccaactgcaacttagaagtaacacaaaccgatcaacagtcagcgtggcacaccagccacgttttgatcaaacacttctgttaccccggactgagtatcaatagactgctcacgcggttgaaggagaaaacgttcgttatccggccaactacttcgagaaacctagtaacgccatggaagttgtggagtgtttcgctcagcactaccccagtgtagatcaggttgatgagtcaccgcattccccacgggtgaccgtggcggtggctgcgttggcggcctgcccatggggaaacccatgggacgctcttatacagacatggtgcgaagagtctattgagctagttggtagtcctccggcccctgaatgcggctaatcccaactgcggagcatacactctcaagccagagggtagtgtgtcgtaatgggcaactctgcagcggaaccgactactttgggtgtccgtgtttcattttattcctatactggctgcttatggtgacaattgagagattgttaccatatagctattggattggccatccggtgactaacagagctattatatatctttttgttgggtttataccacttagcttgaaagaggttaaaactctacattacattttaatactgaacaccgcaaaatgggcggcctggactacaaggacgacgatgacaaggccagctgcgtgcccaggagcggcctgatcctgagctgcatctgcctgtactgcggcgtgctgctgcccgtgctgctgcccaacctgcccttcctgacctgcctgagcatgtccaccctggagagcgtgacctacctgcccgagaagggcctgtactgccagaggctgcccagcagcaggacccacggcggcaccgagagcctgaagggcaagaacaccgagaacatgggcttctacggcaccctgaagatgatcttctacaagatgaagaggaagctggaccacggcagcgaggtgaggagcttcagcctgggcaagaagccctgcaaggtgagcgagtacaccagcaccaccggcctggtgccctgcagcgccacccccaccaccttcggcgacctgagggccgccaacggccagggacagcagaggaggaggatcaccagcgtgcagcctcccaccggcttacaggagtggctgaagatgttccagagctggagcggccccgagaagctgctggccctggacgagctgatcgacagctgcgagcccacacaggtgaagcacatgatgcaggtgatcgagccccagttccagagggacttcatcagcctgctgcccaaggagctggccctgtacgtgctgagcttcctggagcccaaggacctgctgcaggccgcccagacctgcaggtactggaggatcctggccgaggacaacctgctgtggagggagaagtgcaaggaggagggcatcgacgagcccctgcacatcaagaggaggaaggtgatcaagcccggcttcatccacagcccctggaagagcgcctacatcaggcagcacaggatcgacacaaactggaggaggggcgagctgaagagccccagcgggagcggcagcgggagcggcatggacctgggcaagaagctgctggaggccgccagggccggccaggacgacgaggtgaggatcctgatggccaacggcgccgacgtgaacgccagcgacaggggcggaggcacccccttgcacttagctgctgccggaggccaccttgagatcgtggaagtgttgctgaagaggggcgctgatgtgtctgctgctgacttgcacggacagagccctctgcacctggctgccatggttggacacctggagatcgtggaggtgctgctgaagtacggcgccgacgtgaacgctaaggacaccatgggcgccacccccttgcatctggccgccaggtctggacacctggagatcgtcgaggagctgctgaagaacggcgctgacatgaacgcccaggacaagttcggcaagaccaccttcgacatcagcaccgacaacggcaacgaggacctggctgagatcctgcagaagctgtgaaaaaaacaaaaaacaaaacggctattatgcgttaccggcgagacgctacggactta

SEQ ID NO: 48 - RNA, 1897 nt, synthetic construct
  misc_feature 1..1897: note = circular RNA molecule sequence
  source 1..1897: mol_type = other RNA
aaaatccgttgaccttaaacggtcgtgtgggttcaagtccctccacccccacgccggaaacgcaatagccgaaaaaacaaaaacaaaaaaaacaaaaaaacaaaaaaaaaaccaaaacacattaaaacagcctgtgggttgatcccacccacagggcccactgggcgctagcactctggtatcacggtacctttgtgcgcctgttttatacttcctcccccaactgcaacttagaagtaacacaaaccgatcaacagtcagcgtggcacaccagccacgttttgatcaaacacttctgttaccccggactgagtatcaatagactgctcacgcggttgaaggagaaaacgttcgttatccggccaactacttcgagaaacctagtaacgccatggaagttgtggagtgtttcgctcagcactaccccagtgtagatcaggttgatgagtcaccgcattccccacgggtgaccgtggcggtggctgcgttggcggcctgcccatggggaaacccatgggacgctcttatacagacatggtgcgaagagtctattgagctagttggtagtcctccggcccctgaatgcggctaatcccaactgcggagcatacactctcaagccagagggtagtgtgtcgtaatgggcaactctgcagcggaaccgactactttgggtgtccgtgtttcattttattcctatactggctgcttatggtgacaattgagagattgttaccatatagctattggattggccatccggtgactaacagagctattatatatctttttgttgggtttataccacttagcttgaaagaggttaaaactctacattacattttaatactgaacaccgcaaaatgggcggcctggactacaaggacgacgatgacaaggccagccacaggaagcacctgcaggagatccccgacctgagcagcaacgtggccaccagcttcacctggggctgggacagcagcaagaccagcgagctgctgagcggcatgggcgtgagcgccctggagaaggaggagcccgacagcgagaacatcccccaggagctgctgagcaacctgggccaccccgagagccctcccaggaagaggctgaagagcaagggcagcgacaaggacttcgtgatcgtgcggaggcccaagctgaacagggagaacttccccggcgtgagctgggacagcctgcccgacgagctgctgctgggcatcttcagctgcctgtgcctccccgagctgctgaaggtgagcggcgtgtgcaagaggtggtacaggctggccagcgacgagagcctgtggcagaccctggacctgaccggcaagaacctttctggaagcggctctggatctggcatggacctgggcaagaagctgctggaagctgccagggctggacaagacgacgaggtgaggatcctgatggccaacggcgctgacgtgaacgccagcgacaggggcggaggaacccctttgcaccttgctgccgctggaggacacctggagatcgtggaggtgctgctgaagaggggcgccgacgtgagcgccgctgacctgcatggacagagccccctgcacctggccgccatggtgggacaccttgagatcgtggaggtgctgttgaagtacggcgctgacgtgaacgctaaggacaccatgggcgccacccccttgcacctggccgctaggagcggccacctggagatcgtggaggagctgctgaagaacggcgccgacatgaacgcccaggacaagttcggcaagaccaccttcgacatcagcaccgacaacggcaacgaggacctggccgagatcctgcagaagctgtgaaaaaaacaaaaaacaaaacggctattatgcgttaccggcgagacgctacggactta

SEQ ID NO: 49 - RNA, 2416 nt, synthetic construct
  misc_feature 1..2416: note = circular RNA molecule sequence
  source 1..2416: mol_type = other RNA
aaaatccgttgaccttaaacggtcgtgtgggttcaagtccctccacccccacgccggaaacgcaatagccgaaaaaacaaaaacaaaaaaaacaaaaaaacaaaaaaaaaaccaaaacacattaaaacagcctgtgggttgatcccacccacagggcccactgggcgctagcactctggtatcacggtacctttgtgcgcctgttttatacttcctcccccaactgcaacttagaagtaacacaaaccgatcaacagtcagcgtggcacaccagccacgttttgatcaaacacttctgttaccccggactgagtatcaatagactgctcacgcggttgaaggagaaaacgttcgttatccggccaactacttcgagaaacctagtaacgccatggaagttgtggagtgtttcgctcagcactaccccagtgtagatcaggttgatgagtcaccgcattccccacgggtgaccgtggcggtggctgcgttggcggcctgcccatggggaaacccatgggacgctcttatacagacatggtgcgaagagtctattgagctagttggtagtcctccggcccctgaatgcggctaatcccaactgcggagcatacactctcaagccagagggtagtgtgtcgtaatgggcaactctgcagcggaaccgactactttgggtgtccgtgtttcattttattcctatactggctgcttatggtgacaattgagagattgttaccatatagctattggattggccatccggtgactaacagagctattatatatctttttgttgggtttataccacttagcttgaaagaggttaaaactctacattacattttaatactgaacaccgcaaaatgggcggcctggactacaaggacgacgatgacaaggccagcgccggcgagggcgaccagcaggacgccgcccacaacatgggcaaccacctgcccctgctgcccgccgagagcgaggaggaggacgagatggaggtggaagaccaggacagcaaggaggccaagaagcccaacatcatcaacttcgacaccagcctgcccaccagccacacctacctgggcgccgacatggaggagttccacggcaggaccctgcacgacgacgacagctgccaggtgatccccgtgctgccccaggtgatgatgatcctgattcccggccagaccctgcccctccagctgttccacccccaggaggtgagcatggtgaggaacctgatccagaaggacaggaccttcgccgtgctggcctacagcaacgtgcaggagagggaggcccagttcggcaccaccgccgagatctacgcctacagggaggagcaggacttcggcatcgagatcgtgaaggtcaaggccatcggcaggcagaggttcaaggtgctggagctgaggacccagagcgacggcatccagcaggccaaggtgcagatcctgcccgagtgcgtgctgcccagcaccatgagcgccgtgcagctggagagcctgaacaagtgccagatcttccccagcaagcccgtgagcagggaggaccagtgcagctacaagtggtggcagaagtaccagaagaggaagttccactgcgccaacctgaccagctggcccaggtggctgtacagcctgtacgacgccgagaccctgatggacaggatcaagaagcagctgagggagtgggacgagaacctgaaggacgacagcctgcccagcaaccccatcgacttcagctacagggtggccgcctgcctgcccatcgacgacgtgctgaggatccagctgctgaagatcggcagcgccatccagaggctgaggtgcgagctggacatcatgaacaagtgcaccagcagcggctccggcagcggctccggcatggacctgggcaagaagctgctggaggccgccagggccggccaggacgacgaggtgaggatcctgatggccaacggcgccgacgtgaacgccagcgacaggggcggcggcacccccttgcacctggctgctgctggaggccaccttgagatcgtggaggtgctgctgaagaggggcgctgacgtttctgctgctgaccttcatggacagtctcctctgcacctggctgctatggtgggccacctggagatcgtggaggtgctgttgaagtacggcgccgacgtgaacgctaaggacaccatgggcgccacacctttgcacttggctgctaggagcggccacttggagatcgtggaggagttgctgaagaacggcgccgacatgaacgcccaggacaagttcggcaagaccaccttcgacatcagcaccgacaacggcaacgaggacctggccgagatcctgcagaagctgtgaaaaaaacaaaaaacaaaacggctattatgcgttaccggcgagacgctacggactta

SEQ ID NO: 50 - RNA, 1798 nt, synthetic construct
  misc_feature 1..1798: note = circular RNA molecule sequence
  source 1..1798: mol_type = other RNA
aaaatccgttgaccttaaacggtcgtgtgggttcaagtccctccacccccacgccggaaacgcaatagccgaaaaaacaaaaacaaaaaaaacaaaaaaacaaaaaaaaaaccaaaacacattaaaacagcctgtgggttgatcccacccacagggcccactgggcgctagcactctggtatcacggtacctttgtgcgcctgttttatacttcctcccccaactgcaacttagaagtaacacaaaccgatcaacagtcagcgtggcacaccagccacgttttgatcaaacacttctgttaccccggactgagtatcaatagactgctcacgcggttgaaggagaaaacgttcgttatccggccaactacttcgagaaacctagtaacgccatggaagttgtggagtgtttcgctcagcactaccccagtgtagatcaggttgatgagtcaccgcattccccacgggtgaccgtggcggtggctgcgttggcggcctgcccatggggaaacccatgggacgctcttatacagacatggtgcgaagagtctattgagctagttggtagtcctccggcccctgaatgcggctaatcccaactgcggagcatacactctcaagccagagggtagtgtgtcgtaatgggcaactctgcagcggaaccgactactttgggtgtccgtgtttcattttattcctatactggctgcttatggtgacaattgagagattgttaccatatagctattggattggccatccggtgactaacagagctattatatatctttttgttgggtttataccacttagcttgaaagaggttaaaactctacattacattttaatactgaacaccgcaaaatgggcggcctggactacaaggacgacgatgacaaggccagcgcccccaagaagaggcccgagacccagaagaccagcgagatcgtgctgaggcccaggaacaagaggagcaggtcccccttggagctcgagcccgaggccaagaagctgtgcgccaagggcagcggccccagcaggaggtgcgacagcgactgcctgtgggtgggcctggccggcccccagatcctgcccccttgcaggagcatcgtgaggaccctgcaccagcacaagctgggcagggccagctggcccagcgtgcagcagggcctgcagcagagcttcctgcacaccctggacagctacaggatcctgcagaaggccgcccccttcgacaggagggccagcggctccgggagcggcagcgggatggacctgggcaagaagctgctggaagctgctagggctggacaggatgatgaagttaggattttaatggctaatggagctgatgttaatgcctctgacaggggcggaggaacacccttgcatttagccgctgccggcggccacttagagatcgtggaggtgctgctgaagaggggcgctgacgtgagcgctgctgacttgcacggacagagccccttgcacctggccgccatggttggacacctggagatcgtggaggtgctgttgaagtacggcgccgacgtgaacgccaaggacaccatgggcgccacccccttgcacctggccgcccggagcggccacctggagatcgtggaggagctgctgaagaacggcgccgacatgaacgcccaggacaagttcggcaagaccaccttcgacatcagcaccgacaacggcaacgaggacctggccgagatcctgcagaagctgtgaaaaaaacaaaaaacaaaacggctattatgcgttaccggcgagacgctacggactta

SEQ ID NO: 51 - RNA, 1591 nt, synthetic construct
  misc_feature 1..1591: note = circular RNA molecule sequence
  source 1..1591: mol_type = other RNA
aaaatccgttgaccttaaacggtcgtgtgggttcaagtccctccacccccacgccggaaacgcaatagccgaaaaaacaaaaacaaaaaaaacaaaaaaacaaaaaaaaaaccaaaacacattaaaacagcctgtgggttgatcccacccacagggcccactgggcgctagcactctggtatcacggtacctttgtgcgcctgttttatacttcctcccccaactgcaacttagaagtaacacaaaccgatcaacagtcagcgtggcacaccagccacgttttgatcaaacacttctgttaccccggactgagtatcaatagactgctcacgcggttgaaggagaaaacgttcgttatccggccaactacttcgagaaacctagtaacgccatggaagttgtggagtgtttcgctcagcactaccccagtgtagatcaggttgatgagtcaccgcattccccacgggtgaccgtggcggtggctgcgttggcggcctgcccatggggaaacccatgggacgctcttatacagacatggtgcgaagagtctattgagctagttggtagtcctccggcccctgaatgcggctaatcccaactgcggagcatacactctcaagccagagggtagtgtgtcgtaatgggcaactctgcagcggaaccgactactttgggtgtccgtgtttcattttattcctatactggctgcttatggtgacaattgagagattgttaccatatagctattggattggccatccggtgactaacagagctattatatatctttttgttgggtttataccacttagcttgaaagaggttaaaactctacattacattttaatactgaacaccgcaaaatggacctgggcaagaagctgctggaggccgccagggccggccaggacgacgaggtgaggatcctgatggccaacggcgccgacgtgaacgccagcgacaggggcggcggcacccccttgcacctggccgccgccggcggccacctggagatcgtggaggtgctgctgaagaggggcgccgacgtgagcgccgccgacctgcacggccagagccccctgcacctggccgccatggtgggccacctggaaatcgtggaggtgctgctcaagtacggcgccgacgtgaacgctaaggacaccatgggcgccacccccttgcacctggctgccaggagcggccacctggagatcgtcgaggagctgctgaagaacggcgccgacatgaacgcccaggacaagttcggcaagaccaccttcgacatcagcacagataatggcaatgaagatctggctgaaattttacaaaaattaagcggatctgggtctggctctggacctaggaacggcaccgttcacttgtacctgaccaagcccctgtacaccagcgcccccagcctgcagcacctgtgcaggctgaccatcaacaagtgcaccggcgccatctggggcctgcccctccccaccaggctgaaggactacctggaggagtacaagttccaggtgggcagctgaaaaaaacaaaaaacaaaacggctattatgcgttaccggcgagacgctacggactta

SEQ ID NO: 52 - RNA, 1633 nt, synthetic construct
  misc_feature 1..1633: note = circular RNA molecule sequence
  source 1..1633: mol_type = other RNA
aaaatccgttgaccttaaacggtcgtgtgggttcaagtccctccacccccacgccggaaacgcaatagccgaaaaaacaaaaacaaaaaaaacaaaaaaacaaaaaaaaaaccaaaacacattaaaacagcctgtgggttgatcccacccacagggcccactgggcgctagcactctggtatcacggtacctttgtgcgcctgttttatacttcctcccccaactgcaacttagaagtaacacaaaccgatcaacagtcagcgtggcacaccagccacgttttgatcaaacacttctgttaccccggactgagtatcaatagactgctcacgcggttgaaggagaaaacgttcgttatccggccaactacttcgagaaacctagtaacgccatggaagttgtggagtgtttcgctcagcactaccccagtgtagatcaggttgatgagtcaccgcattccccacgggtgaccgtggcggtggctgcgttggcggcctgcccatggggaaacccatgggacgctcttatacagacatggtgcgaagagtctattgagctagttggtagtcctccggcccctgaatgcggctaatcccaactgcggagcatacactctcaagccagagggtagtgtgtcgtaatgggcaactctgcagcggaaccgactactttgggtgtccgtgtttcattttattcctatactggctgcttatggtgacaattgagagattgttaccatatagctattggattggccatccggtgactaacagagctattatatatctttttgttgggtttataccacttagcttgaaagaggttaaaactctacattacattttaatactgaacaccgcaaaatggacctgggcaagaagctgctggaggccgccagggccggccaggacgacgaggtgaggatcctgatggccaacggcgccgacgtgaacgccagcgacaggggcggcggcacccctctgcacctggccgccgccggcggccacctggagatcgtggaggtgctgctgaagaggggcgccgacgtgagcgccgccgacctgcacggccagagccccctgcacctggccgccatggtgggccacctggagatcgtcgaggtgctgctgaagtacggcgccgacgtgaacgctaaggacaccatgggcgccacccctctgcacctggctgccaggagcggccacctggagatcgttgaggagctgctgaagaacggcgccgacatgaacgcccaggacaagttcggcaagaccaccttcgacatcagcaccgacaacggcaacgaggatttagctgaaattttacaaaaattaagcggtagcggatctggaagtggagttaaatgggagagccttggacctgagagcaggggcaggaggaaggtggaccccgaggccctgcaggtgttcaaggaggccaggagcgtgcccaggaccctgctgtgcctctgcagggtggccgtgaggagggccctgggcaagcacaggctgcacctgatccccagcctgcccctccccgaccccatcaagaagttcctgctgcacgagggcagctgaaaaaaacaaaaaacaaaacggctattatgcgttaccggcgagacgctacggactta

SEQ ID NO: 53 - RNA, 1951 nt, synthetic construct
  misc_feature 1..1951: note = circular RNA molecule sequence
  source 1..1951: mol_type = other RNA
aaaatccgttgaccttaaacggtcgtgtgggttcaagtccctccacccccacgccggaaacgcaatagccgaaaaaacaaaaacaaaaaaaacaaaaaaacaaaaaaaaaaccaaaacacattaaaacagcctgtgggttgatcccacccacagggcccactgggcgctagcactctggtatcacggtacctttgtgcgcctgttttatacttcctcccccaactgcaacttagaagtaacacaaaccgatcaacagtcagcgtggcacaccagccacgttttgatcaaacacttctgttaccccggactgagtatcaatagactgctcacgcggttgaaggagaaaacgttcgttatccggccaactacttcgagaaacctagtaacgccatggaagttgtggagtgtttcgctcagcactaccccagtgtagatcaggttgatgagtcaccgcattccccacgggtgaccgtggcggtggctgcgttggcggcctgcccatggggaaacccatgggacgctcttatacagacatggtgcgaagagtctattgagctagttggtagtcctccggcccctgaatgcggctaatcccaactgcggagcatacactctcaagccagagggtagtgtgtcgtaatgggcaactctgcagcggaaccgactactttgggtgtccgtgtttcattttattcctatactggctgcttatggtgacaattgagagattgttaccatatagctattggattggccatccggtgactaacagagctattatatatctttttgttgggtttataccacttagcttgaaagaggttaaaactctacattacattttaatactgaacaccgcaaaatggacctgggcaagaagctgctggaggccgccagggccggccaggacgacgaggtgaggatcctgatggccaacggcgccgacgtgaacgccagcgacaggggcggcggcacccccttgcacctggccgccgccggcggccacctggagatcgtggaggtgctgctgaagaggggcgccgacgtgagcgccgccgacctgcacggccagagccccctgcacctggccgccatggtgggccacctggagatcgtcgaggtgctgctgaagtacggcgccgacgtgaacgctaaggacaccatgggcgccacccccttgcacctggctgccaggagcggccacctggagatcgttgaggagctgctgaagaacggcgccgacatgaacgcccaggacaagttcggcaagaccaccttcgacatcagcacagacaatggaaatgaggatttagctgaaattttacaaaaactgtctggcagcggctctggatctggtaggcttaacttcggcgacgacatccctagcgccctgaggatcgccaagaagaagaggtggaacagcatcgaggagaggaggatccaccaggagagcgagctgcacagctacctgagcaggctgatcgccgccgagagagagagggagctggaggagtgccagaggaaccacgagggcgacgaggacgacagccacgtgagggcccagcaggcctgcatcgaggccaagcacgacaagtacatggccgacatggacgagctgttcagccaggtggacgagaagaggaagaagagggacatccccgactacctgtgcggcaagatcagcttcgagctgatgagggagccctgcatcacccccagcggcatcacctacgacaggaaggacatcgaggagcacctgcagagggtgggccacttcgaccccgtgaccaggagccccctgacccaggagcagctgatccccaacctggccatgaaggaggtgatcgacgccttcatcagcgagaacggctgggtggaggactacggcagctgaaaaaaacaaaaaacaaaacggctattatgcgttaccggcgagacgctacggactta

SEQ ID NO: 54 - RNA, 2038 nt, synthetic construct
  misc_feature 1..2038: note = circular RNA molecule sequence
  source 1..2038: mol_type = other RNA
aaaatccgttgaccttaaacggtcgtgtgggttcaagtccctccacccccacgccggaaacgcaatagccgaaaaaacaaaaacaaaaaaaacaaaaaaacaaaaaaaaaaccaaaacacattaaaacagcctgtgggttgatcccacccacagggcccactgggcgctagcactctggtatcacggtacctttgtgcgcctgttttatacttcctcccccaactgcaacttagaagtaacacaaaccgatcaacagtcagcgtggcacaccagccacgttttgatcaaacacttctgttaccccggactgagtatcaatagactgctcacgcggttgaaggagaaaacgttcgttatccggccaactacttcgagaaacctagtaacgccatggaagttgtggagtgtttcgctcagcactaccccagtgtagatcaggttgatgagtcaccgcattccccacgggtgaccgtggcggtggctgcgttggcggcctgcccatggggaaacccatgggacgctcttatacagacatggtgcgaagagtctattgagctagttggtagtcctccggcccctgaatgcggctaatcccaactgcggagcatacactctcaagccagagggtagtgtgtcgtaatgggcaactctgcagcggaaccgactactttgggtgtccgtgtttcattttattcctatactggctgcttatggtgacaattgagagattgttaccatatagctattggattggccatccggtgactaacagagctattatatatctttttgttgggtttataccacttagcttgaaagaggttaaaactctacattacattttaatactgaacaccgcaaaatggacctgggcaagaagctgctggaggccgccagggccggccaggacgacgaggtgaggatcctgatggccaacggcgccgacgtgaacgccagcgacaggggcggcggcacccccttgcacctggccgccgccggcggccacctggagattgtggaggtgctgctgaagaggggcgccgacgtgagcgccgccgacctgcacggccagagccccctgcacctggccgccatggtgggccacctggagatcgtggaggtgctgctgaagtacggcgccgacgtgaacgctaaggacaccatgggcgccacccccttgcacctcgccgccaggagcggccacctggagatcgtcgaggagctgctgaagaacggcgccgacatgaacgcccaggacaagttcggcaagaccaccttcgacatcagcaccgacaacggcaacgaggacttagctgaaattttacaaaaattaggatctggaagcggatcaggatctgttaatatcagcggccagaacaccatgaacatggtgaaggtgcccgagtgcaggctggccgacgagctgggcggcctgtgggagaacagcaggttcaccgactgctgcctgtgcgtggccggccaggagttccaggcccacaaggccatcctggccgccaggagccccgtgttcagcgccatgttcgagcacgagatggaggagagcaagaagaacagggtggagatcaacgacgtggagcccgaggtgttcaaggagatgatgtgcttcatctacaccggcaaggcccccaacctggacaagatggccgacgacctgctggccgccgccgacaagtacgccctggagaggctgaaggtgatgtgcgaggacgccctgtgcagcaacctgagcgtggagaacgccgccgagatcctgattctggccgacctgcacagcgccgaccagctgaagacccaggccgtggacttcatcaactaccacgccagcgacgtgctggagaccagcggctggaagagcatggtggtgagccacccccacctggtggccgaggcctacaggagcctggccagcgcccagtgccccttcctgggccctcctaggaagaggctgaagcagagctgaaaaaaacaaaaaacaaaacggctattatgcgttaccggcgagacgctacggactta

SEQ ID NO: 55 - RNA, 2101 nt, synthetic construct
  misc_feature 1..2101: note = circular RNA molecule sequence
  source 1..2101: mol_type = other RNA
aaaatccgttgaccttaaacggtcgtgtgggttcaagtccctccacccccacgccggaaacgcaatagccgaaaaaacaaaaacaaaaaaaacaaaaaaacaaaaaaaaaaccaaaacacattaaaacagcctgtgggttgatcccacccacagggcccactgggcgctagcactctggtatcacggtacctttgtgcgcctgttttatacttcctcccccaactgcaacttagaagtaacacaaaccgatcaacagtcagcgtggcacaccagccacgttttgatcaaacacttctgttaccccggactgagtatcaatagactgctcacgcggttgaaggagaaaacgttcgttatccggccaactacttcgagaaacctagtaacgccatggaagttgtggagtgtttcgctcagcactaccccagtgtagatcaggttgatgagtcaccgcattccccacgggtgaccgtggcggtggctgcgttggcggcctgcccatggggaaacccatgggacgctcttatacagacatggtgcgaagagtctattgagctagttggtagtcctccggcccctgaatgcggctaatcccaactgcggagcatacactctcaagccagagggtagtgtgtcgtaatgggcaactctgcagcggaaccgactactttgggtgtccgtgtttcattttattcctatactggctgcttatggtgacaattgagagattgttaccatatagctattggattggccatccggtgactaacagagctattatatatctttttgttgggtttataccacttagcttgaaagaggttaaaactctacattacattttaatactgaacaccgcaaaatgcccaggagggccgagaactgggacgaggccgaggtgggcgccgaggaggccggcgtggaggagtacggccccgaggaggacggcggcgaggagagcggcgccgaggagagcggccccgaagagagcggccccgaggaactgggcgccgaggaggagatggaggccggcaggcccagacccgtgctgaggagcgtgaacagcagggagcccagccaggtgatcttctgcaacaggagccccagggtggtgctgcccgtgtggctgaacttcgacggcgagccccagccctaccccaccctgccccctggcaccggcaggaggatccacagctacaggggccacctgtggctgttcagagacgccggcacacacgatggccttctggttaaccaaacagaattatttgtgccttctctgaatgttgacggacagcctatttttgccaatatcacactgcctgtgtatacactgaaagagaggtgcctgcaggttgtgaggagcctggtgaagcccgagaactacaggagactggacatcgtgaggagcctgtacgaggacctggaggaccaccccaacgtgcagaaggacctggagaggctgacccaggagaggatcgcccaccagaggatgggcgacctggagggcggaggcggcagcgccgccgccatggacctgggcaagaagctgctggaggccgccagggccggccaggacgacgaggtgaggatcctgatggccaatggcgccgacgtgaacgccagcgacaggtggggctggacccctctgcacctggccgcctggtggggccacctggagatcgtggaggtgctgttgaagaggggcgctgatgttagcgccgctgatctgcacggacaaagccccctgcatctggctgccatggtgggccacctggaaattgtggaagtgctgttgaagtacggagctgatgttaacgccaaagataccatgggagctacccctctgcacctggctgccaggagcggccacctcgagatcgtggaggagctgttgaagaacggcgctgacatgaacgcccaggacaagttcggcaagaccaccttcgacatcagcaccgacaacggcaacgaggacctggccgagatcctgcagaagctggtggacggcggcagcgactacaaggacgacgatgacaagtgaaaaaaacaaaaaacaaaacggctattatgcgttaccggcgagacgctacggactta

SEQ ID NO: 56 - RNA, 1432 nt, synthetic construct
  misc_feature 1..1432: note = circular RNA molecule sequence
  source 1..1432: mol_type = other RNA
aaaatccgttgaccttaaacggtcgtgtgggttcaagtccctccacccccacgccggaaacgcaatagccgaaaaaacaaaaacaaaaaaaacaaaaaaacaaaaaaaaaaccaaaacacattaaaacagcctgtgggttgatcccacccacagggcccactgggcgctagcactctggtatcacggtacctttgtgcgcctgttttatacttcctcccccaactgcaacttagaagtaacacaaaccgatcaacagtcagcgtggcacaccagccacgttttgatcaaacacttctgttaccccggactgagtatcaatagactgctcacgcggttgaaggagaaaacgttcgttatccggccaactacttcgagaaacctagtaacgccatggaagttgtggagtgtttcgctcagcactaccccagtgtagatcaggttgatgagtcaccgcattccccacgggtgaccgtggcggtggctgcgttggcggcctgcccatggggaaacccatgggacgctcttatacagacatggtgcgaagagtctattgagctagttggtagtcctccggcccctgaatgcggctaatcccaactgcggagcatacactctcaagccagagggtagtgtgtcgtaatgggcaactctgcagcggaaccgactactttgggtgtccgtgtttcattttattcctatactggctgcttatggtgacaattgagagattgttaccatatagctattggattggccatccggtgactaacagagctattatatatctttttgttgggtttataccacttagcttgaaagaggttaaaactctacattacattttaatactgaacaccgcaaaatggacctgggcaagaagctgctggaggccgccagggccggccaggacgacgaggtgaggatcctgatggccaatggcgccgacgtgaacgccagcgacagaggcggcggcacccctctgcacctggccgccgccggcggacacctggaaattgtggaggtgctgttgaagaggggcgctgatgttagcgccgctgatctgcacggacaaagccccctgcatctggctgccatggtgggccacctggaaattgtggaagtgctgttgaagtacggagctgatgttaacgccaaagataccatgggagctacccctctgcacctggctgccaggagcggccacctcgagatcgtggaggagctgttgaagaacggcgctgacatgaacgcccaggacaagttcggcaagaccaccttcgacatcagcaccgacaacggcaacgaggacctggccgagatcctgcagaagctggtggacggcggcagcgactacaaggacgacgatgacaagtgaaaaaaacaaaaaacaaaacggctattatgcgttaccggcgagacgctacggactta

SEQ ID NO: 57 - protein, 10 aa, synthetic construct
  REGION 1..10: note = linker peptide sequence
LEGGGGSAAA